European Patent Specification EP 3 655 422 B1, published March 29, 2023. Title: Promoter for heterologous expression. Applicant: BASF SE. The sequence listing filed with the application follows.

SEQUENCE LISTING (118 sequences)

SEQ ID NO: 1 - DNA, 27 bp, Artificial Sequence
  PCR-amplification of fragment of pCB56C
aggaagagctcggtacccgacgatcat

SEQ ID NO: 2 - DNA, 37 bp, Artificial Sequence
  PCR-amplification of fragment of pCB56C
gaggagtacgtaaaatctttttgttccattaaagggc

SEQ ID NO: 3 - DNA, 30 bp, Artificial Sequence
  PCR-amplification of fragment of pUB110
gacctctacgtaaccaacatgattaacaat

SEQ ID NO: 4 - DNA, 30 bp, Artificial Sequence
  PCR-amplification of fragment of pUB110
ggatcgagctcccaagaaaaacacgattta

SEQ ID NO: 5 - DNA, 33 bp, Artificial Sequence
  PCR-amplification of fragment of pBR322
ccatgtacgtagtggcacttttcggggaaatgt

SEQ ID NO: 6 - DNA, 30 bp, Artificial Sequence
  PCR-amplification of fragment of pBR322
ccaggatatctgagcaaaaggccagcaaaa

SEQ ID NO: 7 - DNA, 37 bp, Artificial Sequence
  PCR-amplification of fragment of lacI from pZS4-int1
aggccggtacctataaaaataggcgtatcacgaggcc

SEQ ID NO: 8 - DNA, 33 bp, Artificial Sequence
  PCR-amplification of fragment of lacI from pZS4-int1
aactcctctagattaattgcgttgcgctcactg

SEQ ID NO: 9 - DNA, 41 bp, Bacilllus licheniformis
aattgtttggaaatgacaaaaggtatgatatgatattgcat

SEQ ID NO: 10 - DNA, 249 bp, Artificial Sequence
  Synthetic DNA fragment comprising the B.licheniformis promoter of secA gene followed by cloning site and terminator
ctcgagaattgtttggaaatgacaaaaggtatgatatgatattgcatatatcgagaccattttctccagcctgcttttccatgcgggctgccgcttatcgtggtctcaagcttagtgactgagcttggactcctgttgatagatccagtaatgacctcagaactccatctggatttgttcagaacgctcggttgccgccgggcgttttttattggtgagaatccaagctaggttggcgagatttctaga

SEQ ID NO: 11 - DNA, 81 bp, Artificial Sequence
  T5-promoter with lac-operator sites
aaatcataaaaaatttatttgctttgtgagcggataacaattataatagattcaattgtgagcggataacaatttcacaca

SEQ ID NO: 12 - DNA, 289 bp, Artificial Sequence
  Synthetic DNA fragment comprising the T5-promoter with lac-operator sites followed by cloning site and terminator
ctcgagaaatcataaaaaatttatttgctttgtgagcggataacaattataatagattcaattgtgagcggataacaatttcacacaatatcgagaccattttctccagcctgcttttccatgcgggctgccgcttatcgtggtctcaagcttagtgactgagcttggactcctgttgatagatccagtaatgacctcagaactccatctggatttgttcagaacgctcggttgccgccgggcgttttttattggtgagaatccaagctaggttggcgagattggtacc

SEQ ID NO: 13 - DNA, 59 bp, Bacillus licheniformis
atataaaaattactgtttactcatgcttaaacaaggaaattaaagaggagcgttattct

SEQ ID NO: 14 - DNA, 39 bp, Artificial Sequence
  PCR-amplification of fragment of pBS1C
aggccggtctccctagtaaggagtgtcaagaatgtttgc

SEQ ID NO: 15 - DNA, 33 bp, Artificial Sequence
  PCR-amplification of fragment of pBS1C
aggccgtctcgtcgaccgtctagccttgccctc

SEQ ID NO: 16 - DNA, 32 bp, Artificial Sequence
  PCR-amplification of fragment of pMDS003
aagggatccctcgagaattgtttggaaatgac

SEQ ID NO: 17 - DNA, 29 bp, Artificial Sequence
  PCR-amplification of fragment of pMDS003
tcctctagagccaacctagcttggattct

SEQ ID NO: 18 - DNA, 1053 bp, Fusobacterium nucleatum 4HI
atgtataaagtagcaagtctttttgcaggtgtaggtggtatagatttgggttttgaacaaacaggtcattttaaaacagtatgggcaaatgaatatgatgataaagctagggaaacatttagatgtaatttttctaataaattaaatgaaaatgatataagagaagtagatgtacaagaaattcctgatatagacatattgttatcaggatttccttgtacttcatttagtgtagcaggttatagaaaaggctttgaagatgaaaatacaggagatttattttttgaaactttaagaattatagttgcaaaacaacctaaagtaatttttttagaaaatgttaaaaatttacttggtcatgataagggaaagacttttaagataataaaagaagctttagaaaaaaataattataaaataaagtatcaagtattaaatgcaaaagactatggaaatataccacaaaatagggaaagaatctatattgttggttttaagaatgaagaacattttaaaaattttgaatttcctttcccattagaattaactagaaatattgaagatatgcttgaaaaaaataatatagatgaaaaatattattattcaaaagaaaaaaataaattttatgataccttagaaaaagaaataactaatgaaaacacaatatatcagtggcgaagaagatatgtaagagaaaataaaagtaatgtgtgtccaacattaactgcaaatatgggaacaggagggcataatgtccctttaataagagttaaagaaagaataagaaaactaacaccaagagaatgttttaattttcaaggatatcccaaggattttaagctcccagatttagctccttctcacttatataaacaagcaggaaattcagttgtagtgccagttataaaaagaattgcagagaatattttcaaagcattggaagaatttaatgtaagttttgaaataaaagtaataaattatttaaaaagtaaaaatattaatacatatgatgaatttttaaattttattgaagaaaagcaaatgaagttgttt

SEQ ID NO: 19 - DNA, 1053 bp, Artificial Sequence
  Codon-variant of MTase gene of Fusobacterium nucleatum 4HI
atgtataaagtggcatctctgtttgccggtgtaggcggtattgaccttggttttgaacagacaggtcattttaaaactgtctgggcgaatgagtacgatgacaaagcccgcgaaacttttagatgcaacttcagtaacaaactgaatgaaaacgatattcgtgaagtggatgtccaagaaattccggacattgatatcttgctatccgggttcccgtgtaccagcttttctgtcgcaggctaccgcaagggctttgaagatgaaaacacgggagatctgtttttcgaaaccttacggatcattgttgcgaaacagccaaaagttatattccttgaaaacgtgaagaacctgttaggtcatgataaagggaaaaccttcaagattatcaaggaagccttggagaaaaataactataagataaaataccaagtgctgaacgcgaaagactacggcaatatccctcaaaatcgtgagcgcatctatatcgtgggtttcaagaatgaagagcacttcaaaaattttgagttccctttcccgctggagctgacccggaacattgaagatatgctcgaaaagaacaatattgacgaaaaatattactatagcaaagaaaaaaacaaattttatgatacgcttgaaaaagagattaccaacgaaaacacgatctaccagtggcgtcgccgttatgtacgtgaaaacaaaagtaacgtgtgtcccacactgactgccaacatgggcaccggcggacataatgtgccgctgatccgtgttaaagagcgaattcgcaaactgacgccacgcgaatgctttaattttcaggggtatccgaaagattttaaactccccgacttagcaccgtcgcacttatataaacaggcgggcaacagcgtagtcgtgccggttatcaaacgtattgctgagaatatctttaaagcgctcgaagagttcaatgtttcctttgagattaaagtgatcaattacttgaagtcgaaaaacatcaatacctatgatgaattcctgaacttcattgaagagaaacagatgaagctgttc

SEQ ID NO: 20 - DNA, 1053 bp, Artificial Sequence
  Codon-variant of MTase gene of Fusobacterium nucleatum 4HI
atgtataaagtcgcgagtctgttcgcgggagtcggcggaattgatcttggttttgagcagaccggccatttcaaaactgtatgggcgaatgaatatgatgacaaagcccgcgagacgttccgttgtaatttcagcaacaagctgaacgaaaacgatattcgtgaagttgacgtccaggaaatcccggacattgatatattgctttcgggtttcccatgcacatctttcagcgttgcaggttaccgcaaagggttcgaagatgagaacacaggggacttatttttcgagactctgcgtattatcgttgccaagcagcccaaagtgatctttctggagaatgtgaaaaacctgttaggccacgataaagggaaaacttttaaaattatcaaagaagctctggaaaaaaacaattataaaatcaagtaccaagttctgaacgcgaaagactacggtaacatcccgcagaatcgtgaacgaatttatatcgtaggctttaaaaatgaagagcactttaaaaactttgagtttccttttcctttggagttaacccggaacatagaggacatgctcgaaaaaaataacattgatgaaaaatactattactccaaagaaaaaaacaaattttatgacactctggagaaagaaattaccaatgaaaatacgatttatcagtggcgccggcgctatgtgcgcgaaaacaagtctaatgtatgcccaaccctgacggccaacatgggcacgggtggccataacgtgcccctcatccgtgtgaaagaaagaatccgcaaactgaccccgcgcgaatgttttaacttccaaggctatccgaaggattttaaattaccggatcttgccccgagtcatctctacaaacaagcaggcaattccgtggtcgtgccggtgattaagcgtattgcggaaaatatctttaaggcactggaggaattcaacgtgtcgtttgagatcaaagttatcaattacctaaagagcaagaacattaatacctacgatgaatttttgaacttcatcgaggaaaaacagatgaaactgttc

SEQ ID NO: 21 - DNA, 1053 bp, Artificial Sequence
  Codon-variant of MTase gene of Fusobacterium nucleatum 4HI
atgtataaagtggcgagcttgtttgcgggtgtgggtggtattgatttaggttttgaacagaccggtcattttaaaaccgtgtgggcgaacgaatatgatgataaagcccgtgaaacctttcgctgcaactttagtaacaaactgaacgaaaacgatattcgcgaagtggatgtgcaggaaatcccagatattgacattttactgtcgggctttccatgcacgtcgtttagcgtggcgggttatcgcaaagggtttgaagatgaaaacaccggcgatctgttttttgaaacgctgcgcatcattgttgcgaaacagccaaaagtgatctttctggaaaacgttaaaaacctgttgggtcatgataagggcaagacgtttaagattattaaagaagccctggaaaaaaacaactataaaattaagtatcaggtgctgaacgcgaaagactatggcaacattccgcagaaccgtgaacgcatatatatcgttggttttaagaacgaagaacattttaaaaactttgaatttccattcccgctggaactgacgcgcaacatcgaagatatgttggaaaaaaacaacattgatgaaaaatattattattcgaaagaaaaaaacaaattttatgatactctggaaaaagaaattacgaacgaaaataccatttatcaatggcggcgccgctatgtgcgcgaaaacaaaagcaacgtctgcccgaccctgacggcgaacatgggcaccggcggacataacgtaccactgattcgcgttaaagaacgcattcgcaaacttaccccgcgcgaatgctttaactttcagggctatcctaaggattttaagctcccggatctggccccaagtcacctgtataaacaggcgggcaactcggttgtggtcccggttattaaacgcatcgcggagaacatcttcaaagcgttagaagaatttaacgtgagctttgaaattaaagtgattaactatctgaaaagcaaaaacatcaacacctatgatgaatttctgaactttatcgaagaaaagcagatgaagttattt

SEQ ID NO: 22 - DNA, 1011 bp, Bacillus licheniformis
atgacttatcgagtaggtagtatgtttgctgggataggtggaacttgtttagggtttatccaagctggcgctaggattgtctgggcaaatgaaatagacaaaaatgcttgtattacttatagaaattattttggggatgcttacttacaagagggtgacattaacctaatagataaaaactccatacctgaactggacattttgattggaggttttccttgccaagccttctctatagctggctatcgtaaagggtttgaagatgaaaggggaaacgtgttctttcaaatattagaggtattggaagcacaaagaaatgtttatggacacttaccccaagcaataatgcttgagaatgtaaagaacttatttacacatgatagaggtaatacgtacagagtaataaaagaggctttggaagcctttggttataccgtaaaagctgaggttcttaattcaatggaatacggtaacgtgccacaaaacagagagcggatttatattgtaggttttcaagatgagagccaagctgaaaggtttagctttccagacccaattcctttaacaaatcaacttaatgatgtaattgaccgaactcggagagttgataaaagatattattatgatgaaacctctcaatattatgatatgttgcgagaagccatggacagtacagatacaacttatcaaataagacgtatatatgttcgagaaaatagaagcaatgtttgtcctacactgacagcgaatatgggaactggagggcataatgttcctattgtattagactttgaaaataatataagaaaactaacaccagaagaatgcttactattgcaaggtttcccagctgactatcattttccagaaggcatggcaaacactcacaaatataaacaagctggtaactctgttacggtgccagttataagaagaattgccactaatattattagcgtattgaacattggaatgaatataaatcaagaacatgaatatgcaatagctgaa

SEQ ID NO: 23 - DNA, 1011 bp, Artificial Sequence
  Codon-variant of MTase gene of Bacillus licheniformis
atgacttatcgagtaggtagtatgtttgccggtattggtggcacctgtctgggttttattcaggcaggcgcacgtattgtttgggccaatgaaattgataaaaatgcctgcattacctatcgcaattattttggtgatgcctatctgcaagaaggtgatattaatctgattgataagaatagcattccggaactggatattctgattggtggttttccgtgtcaggcatttagcattgccggttatcgtaaaggctttgaagatgaacgtggcaatgtgttttttcagattctggaagtgctggaagcacagcgtaatgtttatggtcatctgccgcaggcaattatgctggaaaatgtgaaaaacctgtttacccatgatcgtggtaatacctatcgcgtgattaaagaagcactggaagcctttggttataccgttaaagccgaagttctgaatagcatggaatatggtaatgttccgcagaatcgcgaacgtatttatattgtgggctttcaggatgaaagccaggcagaacgttttagctttccagatccgattccgctgaccaatcagctgaatgatgtgattgatcgtacccgtcgtgtggataaacgctattattatgatgaaaccagccagtattatgatatgctgcgtgaagcaatggatagcaccgataccacctatcagattcgtcgtatttatgtgcgtgaaaatcgtagcaatgtttgtccgaccctgaccgcaaatatgggcaccggtggtcataatgttccgattgtgctggattttgaaaataatattcgcaaactgacaccggaagaatgtctgctgctgcaaggttttccggcagattatcattttccggaaggtatggccaatacccataaatacaaacaggcaggcaatagcgttaccgttccggttattcgtcgcattgccaccaatattatttccgtgctgaatattggcatgaatattaatcaggaacatgaatacgccatcgccgaa

SEQ ID NO: 24 - DNA, 993 bp, Artificial Sequence
  Truncated variant of Bacillus licheniformis Mtase with deletion of 6 amino acids
atgacttatcgagtaggtagtatgtttgctgggataggtggaacttgtttagggtttatccaagctggcgctaggattgtctgggcaaatgaaatagacaaaaatgcttgtattacttatagaaattattttggggatgcttacttacaagagggtgacattaacctaatagataaaaactccatacctgaactggacattttgattggaggttttccttgccaagccttctctatagctggctatcgtaaagggtttgaagatgaaaggggaaacgtgttctttcaaatattagaggtattggaaggacacttaccccaagcaataatgcttgagaatgtaaagaacttatttacacatgatagaggtaatacgtacagagtaataaaagaggctttggaagcctttggttataccgtaaaagctgaggttcttaattcaatggaatacggtaacgtgccacaaaacagagagcggatttatattgtaggttttcaagatgagagccaagctgaaaggtttagctttccagacccaattcctttaacaaatcaacttaatgatgtaattgaccgaactcggagagttgataaaagatattattatgatgaaacctctcaatattatgatatgttgcgagaagccatggacagtacagatacaacttatcaaataagacgtatatatgttcgagaaaatagaagcaatgtttgtcctacactgacagcgaatatgggaactggagggcataatgttcctattgtattagactttgaaaataatataagaaaactaacaccagaagaatgcttactattgcaaggtttcccagctgactatcattttccagaaggcatggcaaacactcacaaatataaacaagctggtaactctgttacggtgccagttataagaagaattgccactaatattattagcgtattgaacattggaatgaatataaatcaagaacatgaatatgcaatagctgaa

SEQ ID NO: 25 - DNA, 945 bp, Bacillus sp. RFL6
atgttacaaatagcaagtttattcgcaggtgtaggtggaattgatttaggatttgaacaaactggatattttgaaacggtttgggcaaatgaatatgataaaaatgcagctattacctatcaatcaaattttaaaaacaaattaattatagatgatattcgaaatatcaaagtagaagatgttcctgattttgatgttttattatcaggatttccttgtacttcttttagcgtggctggatatagaaaaggctttgaagatgaaaaaagcggagatttattttttgaaactttacgcttgattgtagctaaaaaaccacaagttatatttttagaaaatgttaaaaatcttgtgggtcatgacaacggaaatacctttaaagtcatttatgaagcgttagaaagcaacggatatcatataaaataccaagttctaaacgcaaaagattttgggaatatacctcaaaatagagagcgtatctatattgtaggttttaggaatattgaacactataaaaattttaattttccgatgccacaaccacttacattaacaataaaagatatgataaatctttcagataaactagatgatagattttattatacagaggataaatgttctttttattcacctttacaagaacaaatgacttcagatgaaacaatatatcaatggcgtagaaaatatgtgagagaaaacaaaagtaatgtatgccctacgttaactgcgaacatgggaactggaggacataatgttccattagttaaaacaaaacatggaattagaaagttgactcctagagagtgtttcaattttcaaggttatcctgaagatttcattttacccgaattggctcctacgcatctttataagcaagctggaaattctgttgttgttcctgtcataagacgcatagcagaaaatatttataaatctatgttg

SEQ ID NO: 26 - DNA, 1224 bp, Flavobacterium sp. 4H
atgagtttaaaacagacaataagtattaatgaatttgacggcaaaagctatcaaattagacttgttgaaggtattgaagacaaagccgttttaacacattatcttcataactatagaaatggtgtaaaaaagcattacgaaaaagatgctatttcaactctaaaaaatttcgtagaatataaacaagaggaaactgaattacctattgttgcagaagatgctttgcaacaacttttatttgaagttgaaaacgtaccttttccaactccagaaaattatagctttaaattcattgatttatttgcaggaattggaggatttagattagcgttacaaaatgttggcggaaagtgtgtttttacaagcgaatggaataatgaagctcaaaaaacttatcgagaaaattttggagaagttccgtttggcgacataacaaaagagcgaaataaaaattatattcctgaaaaatttgacattttatgtgcaggttttccttgccaagcattttcaattgctggttatcagaaaggttttgctgacacaagaggaactttattttttgacattgagcaaattgtagaaaaacataaacccaaggttgtatttttagaaaatgtaaaaaaccttgtttctcacgacaatggaaatacatttaaaacaattattgaaacacttgaactaaaattgggttataaaacatttgcaaaagttttaaattcagcaactcacgcaaatgttccgcaaaatcgtgagcgaatttttattgttgcatttgacccaaaacaagtgaaaaattattcaaaattcgagtttcctaaaccaatcaaattaacaaaaacaattcacgactttttggataaagaaaagcaagatgatattttttattacaaaaaagaccatcaatattatcctgaacttgtaaaaacaatgatttcaaaagatacggtttatcaatggagaagagtttatgcaagagaaaacaaaagtaacctttgccctactctaacggcaaatatgggttctggcggacataatgtaccattgattatagacgattttggaattagaaaactaactccaaaagaatgttttgcgttccaaggttatccaatcgaaaaatatattattccaaaacttgcaaatagtaaactttatatgcaagctggaaattctgtaacgacaaatttaattgaaagaattgcaaatcaaataattgaagtttta

SEQ ID NO: 27 - DNA, 951 bp, Lactococcus lactis W39
atgttgaaaattgcttcttttttcgccggagttggcggaattgatttaggttttgaaaatgcaggtttcaaaacaatatatgctaatgaatttgataattatgctgctgatacttttgaaatgaactttgacgttaaggtagaccgacgtgatataaatgatgtacaagctgatgaaataccagattttgatattatgttagcaggttttccttgccaagccttttctattgctggttatcgtcaaggctttaacgatgaacaaggtcgaggtaatcttttttttgaacttgttcgtattttagaaacaaaaaaacctcgtgttgcattctttgaaaatgttaaaaatcttgtttctcacgatagcgggaacacatttagagttatttgttctgagttagaaagactagggtacaagtatctttttcaagtgtttaatgcttctgaatatggaaatatacctcaaaatagagaacgtatctatattgttgctttcaaaaataaaaaagattatgcaaattttgaactaccaaaatctatacctttaaaaacaacgattcacgatgttattgatttttctaaaaaacaagacgataagttctactatacctctgaaaagaataaattttttgatgagttaaaagaaaatatgactaatcacgacactacatatcagtggcgtagagtttatgtaagagaaaacaaaagtaatttagtaccaacactaacggctaatatgggaacaggtgggcataatgtgcctataatccttacatatagcggagatattcgtaaattaacaccaagagaatgctttaacgttcaaggtttcccaaaagaatataaacttccaaaccaaagtaatgggagattatataaacaagcaggaaacagtgttgtagtaccagttatagaaagaattgcaaaaaatcttgcagatactatagtcgaa

SEQ ID NO: 28 - DNA, 1623 bp, Clostridium difficile
atgtataatgttatagatctttttgcaggtgcaggtggtttgagcttaggatttgaaatgactaaaaaatttaatatggtggcttttgtagaaaaaaatgataacgcagcaaaaacataccttgaaaatcatccgagtgttaagcgttattgtgatattaaaagattagattttcaagatatattaaacagtgtcgataagatagatgttgttataggaggaccgccatgtcaaggtttttctaatgctaatagacaaaaaagaaaaattataaatggaaataatgaattagttaagctatatgttgatgctattgataaattaaagccaaatgtatttgtaatggaaaatgtcaaaactatatcttcaaataagcattcattttatttgactaaaaaagataaaaatcatataataaataatttaaaattaaatatttataataaagatagtgttttatatgatagaactgagtatataaatgaattatttaatattattagtatagaagatattgaatcatatattatatcaaatatagacttaaaaaatttgaaaataattattaagaaaaaaaaggatatatgtgattatttaaataaaatatctaattataagaaagtaaaatctaccatagaaaaattggaaacaaggggaaaaatgccaaaatggtatttagaattaataaataaagtaaaaaatatattagaaaatatgttatataatagaaatttatcagatgaacaaatattttatttgaacttattcttggatattcaaaatttatttttaggaatatatgagttaaaatctgaatctgtaattttcgaaaatacacttgatgataataaaattatagctaaaatggatacttacattataatagattatataaatgcatcctttgagtatctaggatatgtattaaatggaagtgcactaaattcaattgattatggagtacctcaaaatagagaaagatttgtattgataggagcaaaaaaagacttcttaaaaaataaaaagatagaaactcctaagcctatagttggagaaaattatgttacagtaagagatgcaataggcgatttagctgaatatgaggcttctaaaggtagtatggattattgttttgaaaaaaatagtaataatattgaaaaagatttttatagaaagataatattggatagcaataaaatatacaatcatgtatgtacagatacaagaaatatcgcactaaaaagatttgaatatataaatcaaggaaataattttcattctttgccagatgagttaaaaggaacttatgctgatccagaaagaactcaaaatactatttataaaagactagtatatgataagccatcagatactgttgtaaatgtaagaaaatctatgtggatacatcctattaaaaacagagctgttagcgcaagagaggcggctagattgcagtcattccctgatagttataagtttttaggtacaaaagattctgtatatcaacagataggaaatgcagtaccacctttattaggtcgagtagtagcagaaaagatattaaatttatttaatgatgaaccaaatgagtatcttagagatgtgtttgaagcactagatgga

SEQ ID NO: 29 - DNA, 1623 bp, Clostridium difficile 630; identical to SEQ ID NO: 28

SEQ ID NO: 30 - DNA, 957 bp, Caldicellulosiruptor kristjanssonii 177R1B
gtgattaaaataagagtagtaagtttgttttctggagttggtggtatttgcttagctttcaaacaagcaggatttgatgtgatttgggcaaatgatattgataagtatgcttgtataacatatagatctaatttcccaacagtagagcttgttgaaggtgatatacaaagtattgattccaataatatacctgaatgtgatatcattacagcaggatttccttgccaacctttttctattgcaggttatcagagaggtctcaatgaccctcgtggaagactattttatgaaattgttcgtatcgttcatgataaaaagccaaaaattatttttctcgaaaatgtaaaaaatcttgtttcacataacaacgggattacctttaaaaatattttaaatgctctggaaaatgagggatactatttaaagtatgctgtgcttaattctttagaatacggtaatgtacctcaaaatagggaaagggtttatatagtaggttttttagataaatcaatgtatgaagcatttaagtttccagaaccagtatcactaacagttactattcacgatattattaagccatgggagaaaaaagacgaaaagtattactacagagaagggaagtattatgaacttctcaaacaaaatgtagatgaccctaatacagtttatcagataaggcgtatatatgtcagaaaaaataagaagggtgtatgtcctactttaactgcaaacatgggtgaaggtggtcataatgttcctatcgtaatggataactatggatttagaaaattgaccccacgagaatgtttcatactacaaggcttcccagaagattttgtactaccttcaggtttagcagattctaagttgtataaacaagcaggtaatgccgttactgtaacagttgtaaagcgtattgcagataaaatattggaaacttgtcttgtaaaatcaata

SEQ ID NO: 31 - DNA, 1218 bp, Clostridium mangenotii LM2
atgactaaaaacaatgatgctgtaagtaccaaaaactatactgtagcaagttttttcggtggagttggcggtattgacttaggatttgaacaagctaagaagttcagtacggtttacattaatgaattcgataaaaatgcacaggagacaatatctataaatttccctagggttagtctagatagacgagatatacatgaagtaagggtagatgaagtgccaagtactgatatagttgccgggggatttccatgtcaagctttctcgatagcagggtatagaaaaggatttgaagatgaaagaggagacctgttttttgaacttttaaggattataaaacatcataagccaaaagttatattcatagagaatgtaaaaaatatggttacacatgatcatggaaatacatttaaggtaataagagaagctttaactttaaatggatactatataaaatggaaagtcataaatggaaaagattatggtgatattcctcaaaatagagaacgtatatatataactggatttttagataaaaatgcttttgatgaatttgaatttccgaataaaatagaactgactaatggattagatacagtaatagattttaaagctaaggtagaggataagtactactatagacaaggtatccaaccattttatgataagctagaagaaactataacatctcaaaattcagtttatcaatggagaaggcaatatgttagagagaacaaaagtggagtagtaccaactctaactgctaacatgggaactggagggcataatgtaccccttattctatcatactatggaataagaaaattgactccaagggaaacttttaatattcaaggatttccaacggattttaaattacctgaaatttcaaatgctcagttatataaacaagcagggaatagtgttgtagtaccagttattaaacgtatagcagaaaatatagctaatgcattagaagaagcagagaataagaatgaaatatataatactgtagaagaaaataataaaaatatacttatatatgtagatatgaaaagcaggtttgaaggagagagctttgtgcaagcctactttgatgaagtttgtgaagctaacgactttgcaattataacagaaattccaattttatcagatgaagaatatctaaagcttgtaaaaagaaatgtatcaaagcgtttttattcattacaaactaag

SEQ ID NO: 32 - DNA, 954 bp, Capnocytophaga ochracea DSM 7271
atgggaaaaagcgttaaattcatagatttatttgcaggggtagggggcttccgctatgctttgcagaatataggggctgaatgtgtcttttcgtcagaatgggacaagttcgctcagcaaacctataagctaaactatggagaagttccttttggcgatattactttacaagaaacgaaagataatattcctaatgaatttgatatactttgcgcaggatttccttgtcaagcattttctatagctggatatcaaaaaggttttgaagatattaggggaacacttttttttgagatagaagaaatagtaaggaagcatcgtcctaaggttatttttttagaaaatgtaaagaacttagtgagtcacgataagggtaaaacatttaaggtaataacgaatatcttagaagagaaattaggttacaagatattttataaagtcctcaatacaatggaatatgctaatattccacaaaatagagagcgtatttttatagtagcttttgatcctaaacaagttcctaattataaagagttccaatttcctgaaaaaattaaacttactaaaacgattcatagctttttagagaaaggaaaacagaatgattatttttattatcagctatctcacaaatacagtccagaacttattaaaatagtaacacgtaaagatactatttatcaatggaggcgtgtgtatgttcgagaaaataagaacaatgtttgtcctactttaacagctaatatgggtacagggggacataatgtaccgattattaaagataattttggtattaggaagttaaccccacgagaatgttttaattttcaaggttatccaaaaggctttatactttctaaagaaatagctatatcaaaattatatatgcaggcagggaactctgtgacaatgcctttaattcaaagagtaagtgaacaaattttgaaagtgtta

SEQ ID NO: 33 - protein, 351 aa, Fusobacterium nucleatum 4HI
MYKVASLFAGVGGIDLGFEQTGHFKTVWANEYDDKARETFRCNFSNKLNENDIREVDVQEIPDIDILLSGFPCTSFSVAGYRKGFEDENTGDLFFETLRIIVAKQPKVIFLENVKNLLGHDKGKTFKIIKEALEKNNYKIKYQVLNAKDYGNIPQNRERIYIVGFKNEEHFKNFEFPFPLELTRNIEDMLEKNNIDEKYYYSKEKNKFYDTLEKEITNENTIYQWRRRYVRENKSNVCPTLTANMGTGGHNVPLIRVKERIRKLTPRECFNFQGYPKDFKLPDLAPSHLYKQAGNSVVVPVIKRIAENIFKALEEFNVSFEIKVINYLKSKNINTYDEFLNFIEEKQMKLF

SEQ ID NO: 34 - protein, 337 aa, Bacillus licheniformis
MTYRVGSMFAGIGGTCLGFIQAGARIVWANEIDKNACITYRNYFGDAYLQEGDINLIDKNSIPELDILIGGFPCQAFSIAGYRKGFEDERGNVFFQILEVLEAQRNVYGHLPQAIMLENVKNLFTHDRGNTYRVIKEALEAFGYTVKAEVLNSMEYGNVPQNRERIYIVGFQDESQAERFSFPDPIPLTNQLNDVIDRTRRVDKRYYYDETSQYYDMLREAMDSTDTTYQIRRIYVRENRSNVCPTLTANMGTGGHNVPIVLDFENNIRKLTPEECLLLQGFPADYHFPEGMANTHKYKQAGNSVTVPVIRRIATNIISVLNIGMNINQEHEYAIAE

SEQ ID NO: 35 - protein, 331 aa, Artificial Sequence
  Truncated variant of Bacillus licheniformis Mtase with deletion of 6 amino acids
MTYRVGSMFAGIGGTCLGFIQAGARIVWANEIDKNACITYRNYFGDAYLQEGDINLIDKNSIPELDILIGGFPCQAFSIAGYRKGFEDERGNVFFQILEVLEAQRPQAIMLENVKNLFTHDRGNTYRVIKEALEAFGYTVKAEVLNSMEYGNVPQNRERIYIVGFQDESQAERFSFPDPIPLTNQLNDVIDRTRRVDKRYYYDETSQYYDMLREAMDSTDTTYQIRRIYVRENRSNVCPTLTANMGTGGHNVPIVLDFENNIRKLTPEECLLLQGFPADYHFPEGMANTHKYKQAGNSVTVPVIRRIATNIISVLNIGMNINQEHEYAIAE

SEQ ID NO: 36 - protein, 315 aa, Bacillus sp. RFL6
MLQIASLFAGVGGIDLGFEQTGYFETVWANEYDKNAAITYQSNFKNKLIIDDIRNIKVEDVPDFDVLLSGFPCTSFSVAGYRKGFEDEKSGDLFFETLRLIVAKKPQVIFLENVKNLVGHDNGNTFKVIYEALESNGYHIKYQVLNAKDFGNIPQNRERIYIVGFRNIEHYKNFNFPMPQPLTLTIKDMINLSDKLDDRFYYTEDKCSFYSPLQEQMTSDETIYQWRRKYVRENKSNVCPTLTANMGTGGHNVPLVKTKHGIRKLTPRECFNFQGYPEDFILPELAPTHLYKQAGNSVVVPVIRRIAENIYKSML

SEQ ID NO: 37 - protein, 541 aa, Clostridium difficile
MYNVIDLFAGAGGLSLGFEMTKKFNMVAFVEKNDNAAKTYLENHPSVKRYCDIKRLDFQDILNSVDKIDVVIGGPPCQGFSNANRQKRKIINGNNELVKLYVDAIDKLKPNVFVMENVKTISSNKHSFYLTKKDKNHIINNLKLNIYNKDSVLYDRTEYINELFNIISIEDIESYIISNIDLKNLKIIIKKKKDICDYLNKISNYKKVKSTIEKLETRGKMPKWYLELINKVKNILENMLYNRNLSDEQIFYLNLFLDIQNLFLGIYELKSESVIFENTLDDNKIIAKMDTYIIIDYINASFEYLGYVLNGSALNSIDYGVPQNRERFVLIGAKKDFLKNKKIETPKPIVGENYVTVRDAIGDLAEYEASKGSMDYCFEKNSNNIEKDFYRKIILDSNKIYNHVCTDTRNIALKRFEYINQGNNFHSLPDELKGTYADPERTQNTIYKRLVYDKPSDTVVNVRKSMWIHPIKNRAVSAREAARLQSFPDSYKFLGTKDSVYQQIGNAVPPLLGRVVAEKILNLFNDEPNEYLRDVFEALDG

SEQ ID NO: 38 - protein, 541 aa, Clostridium difficile 630; identical to SEQ ID NO: 37

SEQ ID NO: 39 - protein, 319 aa, Caldicellulosiruptor kristjanssonii 177R1B
MIKIRVVSLFSGVGGICLAFKQAGFDVIWANDIDKYACITYRSNFPTVELVEGDIQSIDSNNIPECDIITAGFPCQPFSIAGYQRGLNDPRGRLFYEIVRIVHDKKPKIIFLENVKNLVSHNNGITFKNILNALENEGYYLKYAVLNSLEYGNVPQNRERVYIVGFLDKSMYEAFKFPEPVSLTVTIHDIIKPWEKKDEKYYYREGKYYELLKQNVDDPNTVYQIRRIYVRKNKKGVCPTLTANMGEGGHNVPIVMDNYGFRKLTPRECFILQGFPEDFVLPSGLADSKLYKQAGNAVTVTVVKRIADKILETCLVKSI

SEQ ID NO: 40 - protein, 406 aa, Clostridium mangenotii LM2
MTKNNDAVSTKNYTVASFFGGVGGIDLGFEQAKKFSTVYINEFDKNAQETISINFPRVSLDRRDIHEVRVDEVPSTDIVAGGFPCQAFSIAGYRKGFEDERGDLFFELLRIIKHHKPKVIFIENVKNMVTHDHGNTFKVIREALTLNGYYIKWKVINGKDYGDIPQNRERIYITGFLDKNAFDEFEFPNKIELTNGLDTVIDFKAKVEDKYYYRQGIQPFYDKLEETITSQNSVYQWRRQYVRENKSGVVPTLTANMGTGGHNVPLILSYYGIRKLTPRETFNIQGFPTDFKLPEISNAQLYKQAGNSVVVPVIKRIAENIANALEEAENKNEIYNTVEENNKNILIYVDMKSRFEGESFVQAYFDEVCEANDFAIITEIPILSDEEYLKLVKRNVSKRFYSLQTK

SEQ ID NO: 41 - protein, 318 aa, Capnocytophaga ochracea DSM 7271
MGKSVKFIDLFAGVGGFRYALQNIGAECVFSSEWDKFAQQTYKLNYGEVPFGDITLQETKDNIPNEFDILCAGFPCQAFSIAGYQKGFEDIRGTLFFEIEEIVRKHRPKVIFLENVKNLVSHDKGKTFKVITNILEEKLGYKIFYKVLNTMEYANIPQNRERIFIVAFDPKQVPNYKEFQFPEKIKLTKTIHSFLEKGKQNDYFYYQLSHKYSPELIKIVTRKDTIYQWRRVYVRENKNNVCPTLTANMGTGGHNVPIIKDNFGIRKLTPRECFNFQGYPKGFILSKEIAISKLYMQAGNSVTMPLIQRVSEQILKVL

SEQ ID NO: 42 - protein, 408 aa, Flavobacterium sp. 4H
MSLKQTISINEFDGKSYQIRLVEGIEDKAVLTHYLHNYRNGVKKHYEKDAISTLKNFVEYKQEETELPIVAEDALQQLLFEVENVPFPTPENYSFKFIDLFAGIGGFRLALQNVGGKCVFTSEWNNEAQKTYRENFGEVPFGDITKERNKNYIPEKFDILCAGFPCQAFSIAGYQKGFADTRGTLFFDIEQIVEKHKPKVVFLENVKNLVSHDNGNTFKTIIETLELKLGYKTFAKVLNSATHANVPQNRERIFIVAFDPKQVKNYSKFEFPKPIKLTKTIHDFLDKEKQDDIFYYKKDHQYYPELVKTMISKDTVYQWRRVYARENKSNLCPTLTANMGSGGHNVPLIIDDFGIRKLTPKECFAFQGYPIEKYIIPKLANSKLYMQAGNSVTTNLIERIANQIIEVL

SEQ ID NO: 43 - protein, 317 aa, Lactococcus lactis W39
MLKIASFFAGVGGIDLGFENAGFKTIYANEFDNYAADTFEMNFDVKVDRRDINDVQADEIPDFDIMLAGFPCQAFSIAGYRQGFNDEQGRGNLFFELVRILETKKPRVAFFENVKNLVSHDSGNTFRVICSELERLGYKYLFQVFNASEYGNIPQNRERIYIVAFKNKKDYANFELPKSIPLKTTIHDVIDFSKKQDDKFYYTSEKNKFFDELKENMTNHDTTYQWRRVYVRENKSNLVPTLTANMGTGGHNVPIILTYSGDIRKLTPRECFNVQGFPKEYKLPNQSNGRLYKQAGNSVVVPVIERIAKNLADTIVE

SEQ ID NO: 44 - protein, 841 aa, Bacillus licheniformis DSM 13
MLGILNKVFDPTKRTLSRYEKKANEIDALKADIEKLSDEALKQKTIEFKERLEKGETVDDLLVEAFAVVREASRRVTGMFPFKVQLMGGVALHEGNIAEMKTGEGKTLTSTMPVYLNALSGKGVHVVTVNEYLASRDAEEMGKIFEFLGLTVGLNLNSLSKDEKREAYAADITYSTNNELGFDYLRDNMVLYKEQMVQRPLHFAVIDEVDSILIDEARTPLIISGQAAKSTKLYVQANAFVRTLKADQDYTYDVKTKGVQLTEEGMTKAEKAFGIENLFDVRHVALNHHIAQALKAHAAMHKDVDYVVEDGQVVIVDSFTGRLMKGRRYSDGLHQAIEAKEGLEIQNESMTLATITFQNYFRMYEKLAGMTGTAKTEEEEFRNIYNMQVVTIPTNKPIARDDRPDLIYRTMEGKFKAVAEDVAQRYMVGQPVLVGTVAVETSELISRLLKNKGIPHQVLNAKNHEREAQIIEDAGQKGAVTIATNMAGRGTDIKLGEGVKELGGLAVIGTERHESRRIDNQLRGRSGRQGDPGITQFYLSMEDELMKRFGAERTMAMLDRFGMDDSTPIQSKMVSRAVESSQKRVEGNNFDARKQLLQYDDVLRQQREVIYKQRFEVIDSDNLRSIVENMIKASLERAVASYTPKEDLPEEWNLDGLVELVNANFLDEGGVEKSDIFGKEPEEITELIYDRIKTKYDEKEERYGSEQMREFEKVIVLREVDTKWMDHIDAMDQLRQGIHLRAYAQTNPLREYQMEGFAMFENMIAAIEDDVAKFVMKAEIENNLEREEVIQGQTTAHQPKEGDEEKQAKKKPVRKAVDIGRNDPCYCGSGKKYKNCCGRTE

SEQ ID NO: 45 - protein, 901 aa, Escherichia coli K12
MLIKLLTKVFGSRNDRTLRRMRKVVNIINAMEPEMEKLSDEELKGKTAEFRARLEKGEVLENLIPEAFAVVREASKRVFGMRHFDVQLLGGMVLNERCIAEMRTGEGKTLTATLPAYLNALTGKGVHVVTVNDYLAQRDAENNRPLFEFLGLTVGINLPGMPAPAKREAYAADITYGTNNEYGFDYLRDNMAFSPEERVQRKLHYALVDEVDSILIDEARTPLIISGPAEDSSEMYKRVNKIIPHLIRQEKEDSETFQGEGHFSVDEKSRQVNLTERGLVLIEELLVKEGIMDEGESLYSPANIMLMHHVTAALRAHALFTRDVDYIVKDGEVIIVDEHTGRTMQGRRWSDGLHQAVEAKEGVQIQNENQTLASITFQNYFRLYEKLAGMTGTADTEAFEFSSIYKLDTVVVPTNRPMIRKDLPDLVYMTEAEKIQAIIEDIKERTAKGQPVLVGTISIEKSELVSNELTKAGIKHNVLNAKFHANEAAIVAQAGYPAAVTIATNMAGRGTDIVLGGSWQAEVAALENPTAEQIEKIKADWQVRHDAVLEAGGLHIIGTERHESRRIDNQLRGRSGRQGDAGSSRFYLSMEDALMRIFASDRVSGMMRKLGMKPGEAIEHPWVTKAIANAQRKVESRNFDIRKQLLEYDDVANDQRRAIYSQRNELLDVSDVSETINSIREDVFKATIDAYIPPQSLEEMWDIPGLQERLKNDFDLDLPIAEWLDKEPELHEETLRERILAQSIEVYQRKEEVVGAEMMRHFEKGVMLQTLDSLWKEHLAAMDYLRQGIHLRGYAQKDPKQEYKRESFSMFAAMLESLKYEVISTLSKVQVRMPEEVEELEQQRRMEAERLAQMQQLSHQDDDSAAAAALAAQTGERKVGRNDPCPCGSGKKYKQCHGRLQ

SEQ ID NO: 46 - protein, 799 aa, Lactobacillus acidophilus NCFM
MANILKKLYNTDKRELKKFEKYATKVEEHADEMSKLSDEQLQAKTPEFRERIKNGESLDDLLPEAFAVAREGAKRVLGLYPFHVQILGGIALHFGNIAEMMTGEGKTLTATMPVYLNALEGKGVHVVTVNEYLSSRDEEEMGQLYRWLGLTVGLNINSMSPDEKREAYNCDVTYSTNSELGFDYLRDNMVVYKEQMVQRPLNYAIIDEVDSILIDEARTPLIISGEAEQANSDYIRADRFVKTLTEDKSDDDADDDEDHGDYKIDWPTKTISLTRTGIEKACEHFGLKNLYDVENQKLVHHIDQALRANYIMLKDIDYVVQDGEVLIVDSFTGRVMEGRRYSDGLHQAIEAKEGVKIQEESRTQATITYQNFFRMYKKLSGMTGTGKTEEEEFREIYNMQVITIPTNRPIARKDMPDILYPTLDSKFHAVIEEIKKRHAKGQPVLVGTVAIESSERLSHLLDEANIPHAVLNAKNHAKEAQIIMNAGQRGAVTIATNMAGRGTDIKLGPGVKELGGLAVIGTERHESRRIDNQLRGRSGRQGDPGYTRFYLSLEDDLMKRFGGDRVKDFLDRLSDNDDEKVIESRLITRQVESAQKRVEGNNYDTRKQTLQYDDVMRIQREIIYGERMQVIEADKSLKNVLIPMIHRTINSQVDMFTQGDRSQWRLDSLRDFISSSLASEQVTDSIDFKTISVEDLKKKLYDIVEKNFEDKEKALGDPSQMLEFEKVVILRVVDDRWTDHIDAMDQLRQSIGLRGYGQLNPLVEYQDSGYRMFEEMISNIEFDVTRLFMKAEIRQNLSR

SEQ ID NO: 47 - protein, 843 aa, Staphylococcus aureus MW2
MGFLSKILDGNNKEIKQLGKLADKVIALEEKTAILTDEEIRNKTKQFQTELADIDNVKKQNDYLDKILPEAYALVREGSKRVFNMTPYKVQIMGGIAIHKGDIAEMRTGEGKTLTATMPTYLNALAGRGVHVITVNEYLSSVQSEEMAELYNFLGLTVGLNLNSKTTEEKREAYAQDITYSTNNELGFDYLRDNMVNYSEDRVMRPLHFAIIDEVDSILIDEARTPLIISGEAEKSTSLYTQANVFAKMLKQDEDYKYDEKTKAVHLTEQGADKAERMFKVENLYDVQNVDVISHINTALRAHVTLQRDVDYMVVDGEVLIVDQFTGRTMPGRRFSEGLHQAIEAKEGVQIQNESKTMASITFQNYFRMYNKLAGMTGTAKTEEEEFRNIYNMTVTQIPTNKPVQRNDKSDLIYISQKGKFDAVVEDVVEKHKAGQPVLLGTVAVETSEYISNLLKKRGIRHDVLNAKNHEREAEIVAGAGQKGAVTIATNMAGRGTDIKLGEGVEELGGLAVIGTERHESRRIDDQLRGRSGRQGDKGDSRFYLSLQDELMIRFGSERLQKMMSRLGLDDSTPIESKMVSRAVESAQKRVEGNNFDARKRILEYDEVLRKQREIIYNERNSIIDEEDSSQVVDAMLRSTLQRSINYYINTADDEPEYQPFIDYINDIFLQEGDITEDDIKGKDAEDIFEVVWAKIEAAYQSQKDILEEQMNEFERMILLRSIDSHWTDHIDTMDQLRQGIHLRSYAQQNPLRDYQNEGHELFDIMMQNIEEDTCKFILKSVVQVEDNIEREKTTEFGEAKHVSAEDGKEKVKPKPIVKGDQVGRNDDCPCGSGKKFKNCHGK

SEQ ID NO: 48 - protein, 845 aa, Corynebacterium glutamicum DSM 20300
MFGLSKVLRVGEGRAVKRLHKIADQVIALEDKFANLTDEELKAKTAEFKERIAGGEGLDEIFLEAFATAREAAWRVLGQKHYHVQIMGGAALHFGNVAEMRTGEGKTLTCVLPAYLNALEGKGVHVVTVNDYLAKRDAEMMGRVHRYLGLEVGVILSDMRPDERREAYAADITYGTNNELGFDYLRDNMARSLSDLVQRGHNYAIVDEVDSILIDEARTPLIISGPVDGTSQFYNVFAQIVPRMTKDVHYEVDERKKTVGVKEEGVEYVEDQLGIDNLYAPEHSQLVSYLNNAIKAQELFTRDKDYIVRNGEVMIVDGFTGRVLAGRRYNEGMHQAIEAKERVEIKNENQTLATVTLQNYFRLYTKLAGMTGTAETEAAELNQIYKLDVIAIPTNRPNQREDLTDLVYKTQEAKFAAVVDDIAERTEKGQPVLVGTVSVERSEYLSQLLTKRGIKHNVLNAKHHEQEAQIVAQAGLPGAVTVATNMAGRGTDIVLGGNPEILLDIKLRERGLDPFEDEESYQEAWDAELPAMKQRCEERGDKVREAGGLYVLGTERHESRRIDNQLRGRSARQGDPGSTRFYLSMRDDLMVRFVGPTMENMMNRLNVPDDVPIESKTVTNSIKGAQAQVENQNFEMRKNVLKYDEVMNEQRKVIYSERREILESADISRYIQNMIEETVSAYVDGATANGYVEDWDLDKLWNALEALYDPSINWTDLVEGSEYGKPGELSAEDLRTALVNDAHAEYAKLEEAVSAIGGEAQIRNIERMVLMPVIDTKWREHLYEMDYLKEGIGLRAMAQRDPLVEYQKEGGDMFNGMKDGIKEETVRQLFLLRKQFIKQDAEVAD

SEQ ID NO: 49 - protein, 911 aa, Pseudomonas putida GB-1
MFAPLLKKLFGSKNEREVKRMLKTVSIVNAFEEKMVALSDEQLRGKTAEFKERLAKGETLDQLLPEAFAVAREAGKRVMGMRHFDVQLIGGMTLHEGMIAEMRTGEGKTLVGTLAVYLNALSGKGVHVVTVNDYLARRDANWMRPLYEFLGLSVGIVSAFQPPEEKRAAYASDITYGTNNEFGFDYLRDNMAFSQEEKFQRELNFAVIDEVDSILIDEARTPLIISGQAEDSSKLYIEINRLIPRLTQHIEEVEGQVTQEGHFTIDEKSRQVELNEAGHQFIEEMLTQAGLLAEGESLYSAHNLGLLTHVYAGLRAHKLFHRNVEYIVQDGQVLLIDEHTGRTMPGRRLSEGLHQAIEAKENLNIQAESQTLASTTFQNYFRLYTKLSGMTGTADTEAFEFQSIYALNVMVIPPNKPLARKDFNDLVYLTADEKYAAIIADIKESMTKGRPILVGTATIETSEHMSNLLKKEGIDHKVLNAKYHEKEAEIIAQAGAPGALTIATNMAGRGTDILLGGNWEAEVAALENPSAEQIAQIKADWQKRHQQVIEAGGLHVIASERHESRRIDNQLRGRSGRQGDPGSSRFYLSLEDSLMRIFASDRVKNFMKALGMQSGEAIEHRMVTNAIEKAQRKVEGRNFDIRKQLLEYDDVANEQRKVIYHMRNSLLAAENIGDTIVEFRQEVLDATISQHIPPQSLPEQWDVAGLEASLASDFAMKLPIQQWLDEDDHLYEETLREKLLNEITTAYTEKEDQAGIEALRTFEKQILLRVLDDLWKDHLSTMDHLRHGIHLRGYAQKNPKQEYKRESFSLFQELLESIKRDTIRVLSHVQVRREDPIEEEARLRREAEELASRMQFQHAAAPGLESEQLSEEGAEVAVAAAPVRNDQKLGRNEPCWCGSGKKFKHCHGQIE

SEQ ID NO: 50 - protein, 947 aa, Streptomyces coelicolor A3(2)
MSVLSKLMRAGEGKILRKLHRIADQVNSIEEDFADLSDAELRALTDEYKQRYADGESLDDLLPEAFATVREAAKRVLGQRHYDVQIMGGAALHMGYVAEMKTGEGKTLVGTLPAYLNALSGEGVHIVTVNDYLAERDSELMGRVHKFLGLNVGCILANQTPAQRREMYACDITYGTNNEFGFDYLRDNMAWSKDELVQRGHNFAIVDEVDSILVDEARTPLIISGPADQATKWYGDFAKLVTRLKKGEAGNTLKGIEETGDYEVDEKKRTVAIHESGVAKVEDWLGIDNLYESVNTPLVGYLNNAIKAKELFKKDKDYVVLDGEVMIVDEHTGRILAGRRYNEGMHQAIEAKEGVDIKDENQTLATITLQNFFRLYKRHDHDGKEQPGLSGMTGTAMTEAAEFHQIYKLGVVPIPTNRPMVRKDQSDLIYRTEVAKFEAVVDDIEEKHRKGQPILVGTTSVEKSEYLSQQLSKRGVQHEVLNAKQHDREATIVAQAGRKGSVTVATNMAGRGTDIKLGGNPEDLAEAELRQRGLDPEEHIEEWAAALPAALERAEQAVKAEFEEVKELGGLYVLGTERHESRRIDNQLRGRSGRQGDPGESRFYLSLGDDLMRLFKAQMVERVMSMANVPDDVPIENKMVTRAIASAQSQVETQNFETRKNVLKYDEVLNRQREVIYGERRRVLEGEDLQEQIQHFTNDTIDAYVQAETAEGFPEDWDLDRLWGAFKQLYPVKVTVEELEEAAGDRAGLTADYIAESIKDDVREQYEAREKQLGSEIMRELERRVVLSVLDRKWREHLYEMDYLQEGIGLRAMAQKDPLVEYQREGFDMFQAMMDGIKEESVGYLFNLEVQVEQQVEEVPVEDAAPSLDKGAQDAVPAQAGARPEIRAKGLDAPQRRDLHFSAPTVDGEGGVVEGEFTDGEPAQAQSDGLTRAERRKQAKGGRRRKK

SEQ ID NO: 51 - protein, 921 aa, Gluconobacter oxydans 621H
MFARLARALFGSANDRTLKAYQRRVPEINALEPAVQALSDEQLRHKTTEFKERLEKGETLDGLLPEAFAVCREASRRVLGKRHFDVQLIGGMVLHAGRIAEMRTGEGKTLVATLAVYLNALSGKGVHVVTVNDYLARRDAEEMSILYSFLGLTTGVIVPNLSDGERREAYAADITYGTNNEFGFDYLRDNMKYSLADMVQRPFNHAIVDEVDSILIDEARTPLIISGPADDSSDLYRSVDDVVVKLVQEPDVYDKDEKLRSVTLTEHGSHRVEELLAEAGVLQDGGLYDIHNVAVVHHVQQSLRAHTLFTRDVDYIVRDGKVVIIDEFTGRMMDGRRYSDGLHQALEAKEHVEIQQENQTLASITFQNYFRLYPKLSGMTGTAMTEADEFAEIYHLDVVEIPTNLPVRRIDTDDEVYLTAAEKFSAVADLIKEIHETGQPILVGTTSIEKSEYLSHILTQRGIPHNVLNARQHEKEAIIVAQAGAPGAITIATNMAGRGTDIKLGGNIEMLVKASTEGVEDEAQRESVEQNIRAIVEEHHEEVHKAGGLYVIGTERHESRRVDNQLRGRSGRQGDPGNSRFFLSLEDDLIRIFASDRMGAMMQKMGLKEGEAIVHPWLNKALEKAQKRVEARNFDMRKNTLKYDDVMNDQRKEVYAQRREYMATDDLSGVIAELREHTIEDLVHAHIPEKSFAEAWDTEGLTKEVSRILNLDLPIADWAKEDGMDSEGVIERIEAEAAKAQAARTANMGPELMRLIEKQVVLTTFDAVWKEYLHGLDQLRQGIGLRAYGQRDPLNEYKQEAFQMFTAMLDDMRIRVTETMCRIQAVSEPPPFPVINTETSGPSEEPAGLFSQGTTGGDIPAPQPMAGFPSAAPMPPRPQPVPTGAEPDAATLQRWYAETPRNALCPCGSGLKFKHCHGRLA

SEQ ID NO: 52 - protein, 839 aa, Clostridium acetobutylicum DSM 792
MGLLEKIFGTYSDREVKRIIPLVDKIDALDGSMQALSEDELKAKTAEFKQRYENGETLDDLLVEAFAVVREASSRILGLKHFREQIIGGIVLHQGRISEMKTGEGKTLVATLPSYLNAITGKGVHVVTVNDYLAKRDMEWMGQLYQYLGLTTGVIVHDLDQKQRQEAYAADITYGTNNEFGFDYLRDNMVIYKEERVQRPLHFCIVDEVDSILIDEARTPLIISGEGEKSTEFYKVADNFAKMLRKEKDFTIDEKTNSAILTDEGVEKAEKYYHIDNYADPQNMEIQHHTSQALKANYLMKRDKDYMVKEDEVVIVDEFTGRLMEGRRYSDGLHQAIEAKEGVKVQKESKTLATITFQNYFRMYEKLSGMTGTALTEEVEFREIYGLDVVVIPTHRPIARIDAPDIVYKTELGKFKAVVEDIVETNKNGQPVLVGTVSIEKSELLSSLLKKRGVRHQVLNAKYHEQEAEIISHAGEKGMVTIATNMAGRGTDIKLGEGVTDVGGLKIIGTERHESRRIDNQLRGRAGRQGDKGYSRFYVSLEDDLMRIFGSDKLKNMVEKLGLGDDDAIESKMVSSAIENAQKKVEGNNFDIRKTLIQYDDVMNKQREIIYKQRSEVLEGENLKDQIEGMIKDLIYNAVNSHISGVDEELESDIEAILNYLDDICLPRGIVEVEELATMSNDEIKEKLYSLAKEIYERKEEEFSSDQMRELERVILLRVVDTKWMDHIDSMEHLKQGIGLRAYKQQDPTQAYQMEGSDMFEEMVENIKVETVRYLFHVQAERAPERQRVVKETEINYSGPDAGDTKKEPVRRKEKKIGRNDLCPCGSGKKYKDCCGRRA

SEQ ID NO: 53 - DNA, 37 bp, Bacillus atrophaeus
aaattctttggaaataacagaaggtatgatatgataa

SEQ ID NO: 54 - DNA, 37 bp, Bacillus subtilis
aaattctttggaaatggcaaaaggtatgttatgataa

SEQ ID NO: 55 - DNA, 37 bp, Bacillus sp.
aaattctttggaaatagcaaaaggtatgttatgataa

SEQ ID NO: 56 - DNA, 37 bp, Bacillus siamensis
aaattctttggaaataaccaaaggtatgttatgataa

SEQ ID NO: 57 - DNA, 37 bp, Bacillus sp.
aaattctttggaaatgaaagaaggtatggtatgataa

SEQ ID NO: 58 - DNA, 37 bp, Bacillus pumilus
aaattctttggaaatgaaggaaggtatggtatgataa

SEQ ID NO: 59 - DNA, 37 bp, Bacillus mojavensis
aaattctttggaaattagagaaggtatgatatgataa

SEQ ID NO: 60 - DNA, 37 bp, Bacillus subtilis
aaattctttggaaataagagaaggtatgatatgataa

SEQ ID NO: 61 - DNA, 37 bp, Bacillus sp.
aaattctttggaaataacaaaaggtgtgatatgataa

SEQ ID NO: 62 - DNA, 37 bp, Bacillus subtilis
aaattctttggaaataacaaaaggtatgatatgataa

SEQ ID NO: 63 - DNA, 37 bp, Bacillus amyloliquefaciens
aaattctttggaaataacaaaaggtatgttatgataa

SEQ ID NO: 64 - DNA, 37 bp, Bacillus sp.
atatggtttggaaatatcataagatgtgataaaataa

SEQ ID NO: 65 - DNA, 37 bp, Bacillus sp.
aaattctttggaaatcaaggaaggtatggtatgataa

SEQ ID NO: 66 - DNA, 37 bp, Bacillus paralicheniformis
aaattgtttggaaatgacaaaaggtatgatatgatat

SEQ ID NO: 67 - DNA, 37 bp, Bacillus glycinifermentans
aaattgtttggaaatgacaaaaggtgtgatatgatat

SEQ ID NO: 68 - DNA, 37 bp, Bacillus vallismortis
aaattctttggaaataacccaaggtatgatatgataa

SEQ ID NO: 69 - DNA, 43 bp, Shigella flexneri
tcattactgctgtggagtgcgcgctttaatgataagatttgtg

SEQ ID NO: 70 - DNA, 43 bp, Citrobacter sp.
tcattactgctgtggtgcgaacgcattaatggtaatatttgtg

SEQ ID NO: 71 - DNA, 43 bp, Salmonella bongori
tcattactgctgttgcgtgtacgctttaatgataagatttgtg

SEQ ID NO: 72 - DNA, 43 bp, Salmonella enterica
tcattactgctgtagcgcgtacgctttaatgataagatttgtg

SEQ ID NO: 73 - DNA, 43 bp, Citrobacter amalonaticus
tcaatactgctgtagtgcctgcgcattaatgataagatttgtg

SEQ ID NO: 74 - DNA, 43 bp, Escherichia albertii
tcattcctgctgtggatttcaggctttaatgataagatttgtg

SEQ ID NO: 75 - DNA, 43 bp, Escherichia sp.
tcattcctgctgtggacttcgggctttaatgataagatttgtg

SEQ ID NO: 76 - DNA, 43 bp, Escherichia sp.
tcattcgtgctgtggactgcaggctttaatggtaagatttgtg

SEQ ID NO: 77 - DNA, 43 bp, Escherichia sp.
tcattcgtgctgtggactgtaggctttaatgataagatttgtg

SEQ ID NO: 78 - DNA, 43 bp, Escherichia sp.
tcattcgtgctgtggactgcaggctttaatgataagatttttg

SEQ ID NO: 79 - DNA, 43 bp, Escherichia sp.
tcattcgtgctgtggaccgcaggctttaatgataagatttgtg

SEQ ID NO: 80 - DNA, 43 bp, Escherichia sp.
tcattcgtgctgcggactgcaggctttaatgataagatttgtg

SEQ ID NO: 81 - DNA, 43 bp, Escherichia sp.
tcattcgtgctgtggactgcaggctttaatgataatatttgtg

SEQ ID NO: 82 - DNA, 43 bp, Escherichia sp.
tcattcgtgctgtggactgcaggctttaatgataagatttgtg

SEQ ID NO: 83 - DNA, 43 bp, Shigella dysenteriae
tcattcatgctgtgggcttcaggctttaatgataagatttgtg

SEQ ID NO: 84 - DNA, 43 bp, Escherichia sp.
tcattcgtgctgtggagttcaggctttaatgataagatttgtg

SEQ ID NO: 85 - DNA, 43 bp, Escherichia sp.
tcattcatgctgtggacttcaggctttaatgataagatttgtg

SEQ ID NO: 86 - DNA, 43 bp, Escherichia sp.
tcattcgtgctgtggacttcaggctttaatgataaaatttgtg

SEQ ID NO: 87 - DNA, 43 bp, Escherichia sp.
tcattcgtgctgtgggcttcaggctttaatgataagatttgtg

SEQ ID NO: 88 - DNA, 43 bp, Escherichia sp.
tcattcgtgctgtggacttcaggctttaatgataagatttgtg

SEQ ID NO: 89 - DNA, 43 bp, Escherichia sp.
tcattcctgctgtggacttcggcctttaatgataagatttgtg

SEQ ID NO: 90 - DNA, 43 bp, Escherichia sp.
tcattcctgctgtggacttcaggctttaatgataagatttgtg

SEQ ID NO: 91 - DNA, 43 bp, Escherichia sp.
tcattcctgctgtggacttcaggctttaatggtaagatttgtg

SEQ ID NO: 92 - DNA, 43 bp, Citrobacter freundii
tcattactgctgtggagcgtacgctttaatgataagattcgtg

SEQ ID NO: 93 - DNA, 43 bp, Citrobacter sp.
tcattactgctgtggagcgtacgctttaatggtaatatttatg

SEQ ID NO: 94 - DNA, 43 bp, Citrobacter freundii
tcattactgctgtggtgcgaacgcattaatggtaagatttgtg

SEQ ID NO: 95 - DNA, 43 bp, Citrobacter koseri
tcattactgctgtagagcgtacgctttaatggtaagatttgtg

SEQ ID NO: 96 - DNA, 43 bp, Citrobacter sp.
tcattactgctgtagagcgtacgctttaatggtaatatttgtg

SEQ ID NO: 97 - DNA, 43 bp, Citrobacter youngae
tcattactgctgtggagcgtacgctttaatggtaatatttgtg

SEQ ID NO: 98 - DNA, 43 bp, Escherichia fergusonii
tcattactgctgtggaatacgggctttaatgataagatttgtt

SEQ ID NO: 99 - DNA, 65 bp, Bacillus pumilus
aaatatggacctgtcaaacttttggacatgccgaaaaattgcatgaaatagaggagcgttattat

SEQ ID NO: 100 - DNA, 69 bp, Bacillus subtilis
atacatgggctagtaaattatttatacatgcctgcacatcaggcatgtgaagatagaggagcgttataa

SEQ ID NO: 101 - DNA, 57 bp, Bacillus glycinifermentans
gaaaattactgtttgcctggctaataaacaaggaaatttacagaggagcgttattct

SEQ ID NO: 102 - DNA, 39 bp, Corynebacterium glutamicum
atcatctttccgtatcgctatttataaggacgactactc

SEQ ID NO: 103 - DNA, 52 bp, Citrobacter freundii
aatggttttgcatttgtaaccccaaacgcagggtatatcaggtggcaataac

SEQ ID NO: 104 - DNA, 46 bp, Salmonella enterica
gttttgattccgtaagcccatgaagggcatatcaggtggcaatgac

SEQ ID NO: 105 - DNA, 29 bp, Escherichia albertii
acgttgaatacgatcgggatggcaataac

SEQ ID NO: 106 - DNA, 37 bp, Staphylococcus saprophyticus
gtaagcgaagagttaaaaagctaaaggagcgaacaga

SEQ ID NO: 107 - DNA, 40 bp, Staphylococcus epidermidis
gtaagccaaacagtttttagttaaaggagcgacgcgtgca

SEQ ID NO: 108 - DNA, 50 bp, Bacillus megaterium
gatagttgatggataaacttgttcacttaaatcaaagggggaaatgtaat

SEQ ID NO: 109 - DNA, 50 bp, Artificial Sequence
  Artificial 5'UTR including a RBS/Shine Dalgarno sequence
atcaagcaaagggcaaggtgtcctagtaaggtcgacaaggaggtctaatt

SEQ ID NO: 110 - DNA, 75 bp, Artificial Sequence
  Artificial 5'UTR including a RBS/Shine Dalgarno sequence
agttactagtagcggccgctgcagtccggcaaaaaagggcaaggtgtcctagtaaggtcgacaggaggactctct

SEQ ID NO: 111 - DNA, 48 bp, Artificial Sequence
  Artificial 5'UTR including a RBS/Shine Dalgarno sequence
gtggaattgtgagcggataacaattcccaattaaaggaggaaggatca

SEQ ID NO: 112 - DNA, 42 bp, Artificial Sequence
  Artificial 5'UTR including a RBS/Shine Dalgarno sequence
aattgtgagcggataacaattaagcttaaggaggtgtatcta

SEQ ID NO: 113 - DNA, 25 bp, Artificial Sequence
  Artificial 5'UTR including a RBS/Shine Dalgarno sequence
actagagaaaggtggtgaatactag

SEQ ID NO: 114 - DNA, 47 bp, Artificial Sequence
  Artificial 5'UTR including a RBS/Shine Dalgarno sequence
aatttgaaaattatgtattatgtgaataaagaggaggagagtgagat

SEQ ID NO: 115 - DNA, 23 bp, Artificial Sequence
  Artificial 5'UTR including a RBS/Shine Dalgarno sequence
aaaattagctagggggaataatt

SEQ ID NO: 116 - DNA, 45 bp, Artificial Sequence
  Artificial 5'UTR including a RBS/Shine Dalgarno sequence
aacggcattgctagacggttacaagaaggaggacgaataattata

SEQ ID NO: 117 - DNA, 44 bp, Artificial Sequence
  Consensus sequence for SecA promoter from Bacillus
  unsure 2 .. 2: All occurrences of k indicate one of the following nucleotides: G, T
  unsure 3 .. 3: All occurrences of n indicate one of the following nucleotides: A, C, G, T
  unsure 13 .. 24: All occurrences of n indicate one of the following nucleotides: A, C, G, T; this sequence segment can be from 8 to 12 nucleotides long
  unsure 25 .. 25: All occurrences of r indicate one of the following nucleotides: A, G
  unsure 27 .. 27: All occurrences of r indicate one of the following nucleotides: A, G
  unsure 30 .. 30: All occurrences of n indicate one of the following nucleotides: A, C, G, T
  unsure 33 .. 33: All occurrences of w indicate one of the following nucleotides: A, T
  unsure 34 .. 34: All occurrences of r indicate one of the following nucleotides: A, G
  unsure 38 .. 38: All occurrences of w indicate one of the following nucleotides: A, T
  unsure 39 .. 44: All occurrences of n indicate one of the following nucleotides: A, C, G, T; this sequence segment can be from 4 to 6 nucleotides long
tkntttggaaatnnnnnnnnnnnnrtrtgntawratawnnnnnn

SEQ ID NO: 118 - DNA, 48 bp, Artificial Sequence
  Consensus sequence for SecA promoter from Enterobacter
  unsure 4 .. 4: All occurrences of w indicate one of the following nucleotides: A, T
  unsure 6 .. 6: All occurrences of m indicate one of the following nucleotides: A, C
  unsure 7 .. 7: All occurrences of n indicate one of the following nucleotides: A, C, G, T
  unsure 13 .. 13: All occurrences of y indicate one of the following nucleotides: C, T
  unsure 14 .. 26: All occurrences of n indicate one of the following nucleotides: A, C, G, T; this sequence segment can be from 11 to 13 nucleotides long
  unsure 33 .. 33: All occurrences of r indicate one of the following nucleotides: A, G
  unsure 37 .. 37: All occurrences of d indicate one of the following nucleotides: A, G, T
  unsure 41 .. 41: All occurrences of y indicate one of the following nucleotides: C, T
  unsure 42 .. 42: All occurrences of d indicate one of the following nucleotides: A, G, T
  unsure 44 .. 48: All occurrences of n indicate one of the following nucleotides: A, C, G, T; this sequence segment can be from 4 to 5 nucleotides long
tcawtmntgctgynnnnnnnnnnnnnttaatgrtaadattydtnnnnn